European Patent Application EP 4 403 636 A1, published July 24, 2024. Title: RECOMBINANT MICROORGANISM WITH CONTROLLED PRODUCTION ABILITY OF POLYOL AND VISCOUS POLYMER. Applicant: GS CALTEX CORPORATION. The sequence listing filed with the application follows.

SEQUENCE LISTING (40 sequences)

SEQ ID NO: 1 - DNA, 1435 bp, Bacillus licheniformis
atgaaagaaaatattgattttagagaactgattgcaatcttgcgaaaaagaacggttcttattctcgttttgacaataggtgtaacattgacgaccggaatcattcagttctatgtgctgacacctgtctatcaggcatcgacgcagatcttggtgcatcaagtaggggagaaaaaggggagcgccacatacagcgatattcaaatcaatcttcaatacacacggacattccaagcgcttttgaaaaacccggtgattttggagcaagtcaagagagagcttgatttaccttactctgcgggccggttgggtgaaaaaattgcaacgagcagtgaaagcgaatctgagattataaatatttcggtccaagatgaaaatcagaaacgggcggccgatatagcgaacactttaactgcggtgctcaaaaaagagattaagcaaattatgaacaccgatcgggtaaccgtcctgtcaaaagccgaaatagtcgattcgccgacacctgtcagaccgaattacaaaatgaatattttgctggcattcggcgccgcattaatgaccggaatcgctttggcgttctttttggactttatcgatgatacggttgcaagaccgtctcaagtcgaaaaggaagcgggattcatttatttgggaagtattgagcaaatgaagcataaaaaaagtctgtttcgcggggaccccgatatgaatatccgcgtaaaagcaggaaggagtgagccgcttgggtattagaaaaaaacgctctcgcaaatatcaatcggcgcttgtcgcattgcatcagccgaacacgccgatcgtcgaacagtatcggacgatcaggacgaacattgagttttcatcatttgagaagccgttcaagtcattgctcattacatcgggcctgccgggagaaggcaaatcattctcggcttcaaacttggcgatcgtattttcgcaacaggaaaaaaaggtccttttgatcgacgcagatttaagaaagccgacgatccataaaatttttgagctcgataaccattcaggcgtcacaaatgtattaatgaaaaaatcgacgctggaaaatgtcgtccagcaaagccaggcggaaaatctccatgtgctgacaagcggtccgattcctccgaatccgtccgagcttttgtcgtcgcaggcgatggaggacctgcttgcggaagcgtacgaccaatacgatttagtcatccttgattcgccgccgcttttgccggtcgcagacgcgcaaatattggcgaatcaggtggatggaagcattcttgtcatcctcagcggaaaaacaaagcttgataacgcgatcaagtctcgggacgcgctgaattcttccaaaagcgaactgctcggcgccgtgctgaacgggcggaaagtgaagaaagcgcgccaatataattacgcaaccatgtaa

SEQ ID NO: 2 - DNA, 484 bp, Bacillus licheniformis
gtacaagatgggttctccactcatcttcctgctcagtccggcgataaaggatcacttcggtatcaaacaattcctttaattcgactttcagcgcccgggagatttttttcaggaattcgactgacggatttctgtgaacgccgcgttcaattttgcttaaatatgattttgatacgcctgctatatcagcaagctggttaatggagtagccttttctctttctgtacattcggatgactcttccgatcatactgaatcctccccttcccttgccattcatataaaacgctttcctgttcattataagaaataatttgttctttataaaattcaaaaatttaagatatcgacagaaaataaaagaaaacgaacgaatttgttctctaaaaagaactatatagctaaattcagcatttttcaattcaaattttttcttttataatccaatcattaacaaacggcattcctgaggaggcagtcaagc

SEQ ID NO: 3 - DNA, 39 bp, Artificial Sequence
  nucleotide sequence of primer for amplifying homologous region 1 of epsAB
agacagggccaacgaggccgtacaagatgggttctccac

SEQ ID NO: 4 - DNA, 33 bp, Artificial Sequence
  nucleotide sequence of primer for amplifying homologous region 1 of epsAB
agccgcttcataagagcttgactgcctcctcag

SEQ ID NO: 5 - DNA, 728 bp, Bacillus licheniformis
tcttatgaagcggctgcagccgctttaggtgatgtctccttgcctttaccgatggaggcactcggctctaccgtgggcagactacctgtctgccttagacgcaagtcgtcgatggcggggcgtgaggacgggttaaatgcccatctttatttaatttacgtgctcggtttaaatttgaaaatcgcccgtatctttttagctcatgggattttgccctgaaagatcctatcagctagaaagatacattaggaggtaggaaattgacatatcggagaaggctttccattattaccgcactcgattcgtacttggttttgctgtccatctttatcggatatcagctgattttgccatcatatgatttatacccttcggaaatgctgctgatgacttcactgatactgcttggcgctcagcatttattcgcccattgcttccacctttataaaaaagtatgggagtatgcaagcatcggtgaattgtatgtgctgcttaaatcgattacattgtcccatcttgtgacggcggccctcgagctgtttttctttcaaaacgttccggttcgtcttttatgtttaagctggctgttccagctcattttgatcggcggatcgcggatgatgtggcgcatcatcagggaacaggtgaacaaagaaagcaaaggatctctaagggcgcttatcatcggagcgggctctgccggcagtttgattgcaaaacagcttgtg

SEQ ID NO: 6 - DNA, 32 bp, Artificial Sequence
  nucleotide sequence of primer for amplifying homologous region 2 of epsAB
aggaggcagtcaagctcttatgaagcggctgc

SEQ ID NO: 7 - DNA, 38 bp, Artificial Sequence
  nucleotide sequence of primer for amplifying homologous region 2 of epsAB
agacagggccttattggccgtcacaagatgggacaatg

SEQ ID NO: 8 - DNA, 1212 bp, Artificial Sequence
  nucleotide sequence of DNA fragment comprising homologous region 1 and 2 of epsAB
gtacaagatgggttctccactcatcttcctgctcagtccggcgataaaggatcacttcggtatcaaacaattcctttaattcgactttcagcgcccgggagatttttttcaggaattcgactgacggatttctgtgaacgccgcgttcaattttgcttaaatatgattttgatacgcctgctatatcagcaagctggttaatggagtagccttttctctttctgtacattcggatgactcttccgatcatactgaatcctccccttcccttgccattcatataaaacgctttcctgttcattataagaaataatttgttctttataaaattcaaaaatttaagatatcgacagaaaataaaagaaaacgaacgaatttgttctctaaaaagaactatatagctaaattcagcatttttcaattcaaattttttcttttataatccaatcattaacaaacggcattcctgaggaggcagtcaagctcttatgaagcggctgcagccgctttaggtgatgtctccttgcctttaccgatggaggcactcggctctaccgtgggcagactacctgtctgccttagacgcaagtcgtcgatggcggggcgtgaggacgggttaaatgcccatctttatttaatttacgtgctcggtttaaatttgaaaatcgcccgtatctttttagctcatgggattttgccctgaaagatcctatcagctagaaagatacattaggaggtaggaaattgacatatcggagaaggctttccattattaccgcactcgattcgtacttggttttgctgtccatctttatcggatatcagctgattttgccatcatatgatttatacccttcggaaatgctgctgatgacttcactgatactgcttggcgctcagcatttattcgcccattgcttccacctttataaaaaagtatgggagtatgcaagcatcggtgaattgtatgtgctgcttaaatcgattacattgtcccatcttgtgacggcggccctcgagctgtttttctttcaaaacgttccggttcgtcttttatgtttaagctggctgttccagctcattttgatcggcggatcgcggatgatgtggcgcatcatcagggaacaggtgaacaaagaaagcaaaggatctctaagggcgcttatcatcggagcgggctctgccggcagtttgattgcaaaacagcttgtg

SEQ ID NO: 9 - DNA, 3001 bp, Bacillus licheniformis
atgtgggtaatgctattagcctgtgtgatcgttgttgggatcggcatttatgaaaaaaggcgccaccagcaaaatatcgatgcgctgcctgtccgagtgaacatcaacggtatacgcggaaagtccacggtgacaagattaacaacagggatattaatcgaagcaggctacaaaacagtaggaaaaacaaccgggacagacgcaaggatgatttattgggacacaccggaagagaagccgatcaaaagaaagccgcaagggccgaatatcggagagcagaaggaggttatgaaagaaacggtggaaagaggggccaatgcgattgtcagtgagtgcatggccgttaatcctgattaccaaatcatctttcaggaagaattgcttcaggctaatatcggcgtgatcgtgaacgtgctggaggatcacatggatgtgatgggaccgactttggatgaaatcgcagaagcattcacagcaaccattccttataatggacatttggttattactgatagtgagtataccgatttctttaagcaaattgcaaaagaaaggaacacaaaagtcatcgtcgcagacaattctaaaataacagatgaatacctcagacagtttgagtacatggtattccctgataatgcgtctcttgcgctcggtgtagctcaagcgttgggcattgacgaagaaaccgcctttaaaggcatgctgaatgcgccgcctgatccgggagccatgagaattctgccgctgatgaacgccaagaatcccggacatttcgtcaacggttttgcggccaatgacgcagcttccactttaaacatttggaagcgtgtaaaagaaataggctatcctacggatcagccgatcgtcattatgaactgccgcgccgacagggtagacagaacacagcagtttgcggaagatgtccttccttatattgaagcaagtgaacttgtgctgattggagaaacaacagagccgatcgtcaaagcatatgaagcaggcaaaattcctgcggacaagctgtttgattttgagcacaaatcaacggaagaaatcatgttcatgctgaaaaacaagcttgagggccgcgttatttacggagtcggaaatatccacggagcagcggagcctctcattgaaaaaatacaagattacaagattaagcagctcgttagctaggaggaagaaaacacaatgtttggatcagatttatatatcgccctcattttaggagtcttactcagtttgatttttgcggagaaaacgggaattgtaccagccggcctcgtcgtaccgggttatttgggacttgtcttcaatcagccgattttcatgctgctcgttctttttgtcagtttgctgacgtatgtcatcgtgaaattcggactttccaaaattatgattctatacggacgcagaaaattcgcagcaatgctgattacgggaattcttttgaaaatcggttttgattttatatatccggtgatgccgtttgagattgccgaattcaggggaatcggaatcatcgtgccggggctgatcgccaataccattcaaagacagggattaacgattacgcttggaagtacgcttttattgagcggagcaacattcgtcattatgtatgcttactatctaatctaaagttaggtgtgtcaaatcgatgaaaaaacaactgaactttcaggaaaaactgctgaagttgacgaagcaggagaaaaagaaaacaaacaagcacgtctttatcgtattgcccgttattttctgtttaatgtttgtctttacttgggtcggaagcgccaaaactccttcgcaaatggacaaaaaagaagatgccaagcttacagctacttttgttggcgatatcatgatgggaagaaacgtagaaaaagtgacaaacttgcacggttcggaaagtgtcttcaaaaatgtgaagccgtactttaatgtgtcagattttatcacaggaaactttgaaaaccctgtaaccaatgcaaaggactatcaagaggcagaaaagaacatccatctgcaaacgaatcaagaatcagtcgaaacattgaaaaagctgaacttcagcgtactgaattttgccaacaaccatgcgatggactacggggaagacggtttgaaggatacgctcaataaattttcaaatgagaatctggagcttgtcggagcaggaaataatcttgaagacgcgaaacagcacgtatcctatcagaatgtgaacggcgtaaaaattgcaacgctcggttttacagacgtctacacaaagaactttacagccaaaaagaacagaggcggagtgctgccgctcagtccgaaaatctttattccaatgattgcggaagcatcgaaaaaagcggatcttgtccttgtccatgtgcactggggacaagaatatgacaatgaaccgaacgacagacagaaggatctggccaaggcgattgcagatgccggagcagatgtcatcatcggcgctcatccccatgttctcgaaccgatcgaagtgtataacggtactgtgattttctacagcctcggcaactttgtatttgatcagggctggtcaagaacacgggacagcgcgcttgtacaataccatttaatgaatgacggcaaagggcgttttgaggtaacgcctctcaacattcgcgaagcaacgccgacgcctttaggcaagagcgacttcttaaaacgaaaagcgatcttccgtcaattgacaaaaggaacaaacctcgactggaaagaagagaacggaaaattaacgtttgaagtcgatcatgcggacaagctgaaaaaataataaaaacggagtggtgaacaaatgaaatttgtcagagccatttggccgttcgtaggtttagttttgatcattgcattcatgtctgctttcaagtattctgatgaattgtcaaacgatgaaaaagctaaaatctctacggagatccaaaaagtgaatcagcaggatcaaacaacagaaaacaagcaataa

SEQ ID NO: 10 - DNA, 792 bp, Bacillus licheniformis
aagccttctcctctctatttgtgtaaccgtttacataaagattatcacgatccatttaaaatcacaataaaaaaatggatgaacactgaaattttagaccgggctgggatatcgagacatatataggggcgtttaatggcgaatacagtaacaatgagaatagtaagaaaaattaaaaatgttaaagtttgatgaattatcattgaaaaaaattaatggctttttaaatcctaggattttaacctaaaatctgaagaaataaggtggatcgaacgactcacaaaatatttggatttgtcaatgaatcccgctttatgctaaaagagattttcattttttgatagatggtctgattgtcataggacggatttgttttgaagagggaacattggtgactttttaacctgttcgaaaagagcgaaaatactaaaagaaaagagagatcccggctgacagcccatttaaaggggattgcggacgggggaaaaaagagatcctgaatccatccttcaacctttcatctgaaatagggagaaaagtacaaaaatcataatgtcgaattttgaaagcgcatacttaaaacgctgacaaaaatctgataggaattaagaactttcgatttccaaaaatatcaataaaaagataggcattaatgactcgggcgaggtgatctttgtcacggaaaatttcgtcgtcttctgttacataatgccgattgtgatttcatagtgaacctatatactgatgaatgaatttacatatcagattccaagaaggagatgtagacaaaca

SEQ ID NO: 11 - DNA, 46 bp, Artificial Sequence
  nucleotide sequence of primer for amplifying homologous region 1 of pgsBCAE
agacagggccaacgaggccaagccttctcctctctatttgtgtaac

SEQ ID NO: 12 - DNA, 40 bp, Artificial Sequence
  nucleotide sequence of primer for amplifying homologous region 1 of pgsBCAE
cggcactctcttttgcactgtgtttgtctacatctccttc

SEQ ID NO: 13 - DNA, 735 bp, Bacillus licheniformis
cagtgcaaaagagagtgccgccggcgctctcttttttgtgtgctgatcccggttataaaagacctgtgaaaagcgaccggtttgaaagggaaacacgacaattttcttaaccggtcagtgtataaagttttatagaaaatcaggaggatatatacatggttttggggttcatgtttattgtattcttttgaagggaataaaaactgacaaatttcgactgaagcaaaatttgaaaatgcatcaccttaccaattcgggatgggaaccgcacctcatgttcatgacctctttagaatatttcccttcatctttttaatctgcgcttaggtgaaaaagctgatcatgctgtgctgagcgtttcttctcgctatgacgctgctgtacatgcaaaaaaagtcctttaaatatcccagttgaatgacgatgaaagaggaaagaagaggaggaacagatcaattgataaaaaaagcggcaaacaaaaagttggttttgttttgtggaattgcggtgctttggatgtctttatttttaacgaatcataatgatgtacgcgccgatacgatcggcgagaaaatagcggaaactgccagacagcttgagggtgcgaaatacagctacggcggagagaagccgaaaacggggtttgactcgtcaggctttgtgcaatatgtgtttcaatcgctcgatattacgcttccgagaacggtaaaggaacaatcgactcttgggagcagt

SEQ ID NO: 14 - DNA, 40 bp, Artificial Sequence
  nucleotide sequence of primer for amplifying homologous region 2 of pgsBCAE
gaaggagatgtagacaaacacagtgcaaaagagagtgccg

SEQ ID NO: 15 - DNA, 43 bp, Artificial Sequence
  nucleotide sequence of primer for amplifying homologous region 2 of pgsBCAE
agacagggccttattggccactgctcccaagagtcgattgttc

SEQ ID NO: 16 - DNA, 1527 bp, Artificial Sequence
  nucleotide sequence comprising homologous region 1 and 2 of pgsBCAE
aagccttctcctctctatttgtgtaaccgtttacataaagattatcacgatccatttaaaatcacaataaaaaaatggatgaacactgaaattttagaccgggctgggatatcgagacatatataggggcgtttaatggcgaatacagtaacaatgagaatagtaagaaaaattaaaaatgttaaagtttgatgaattatcattgaaaaaaattaatggctttttaaatcctaggattttaacctaaaatctgaagaaataaggtggatcgaacgactcacaaaatatttggatttgtcaatgaatcccgctttatgctaaaagagattttcattttttgatagatggtctgattgtcataggacggatttgttttgaagagggaacattggtgactttttaacctgttcgaaaagagcgaaaatactaaaagaaaagagagatcccggctgacagcccatttaaaggggattgcggacgggggaaaaaagagatcctgaatccatccttcaacctttcatctgaaatagggagaaaagtacaaaaatcataatgtcgaattttgaaagcgcatacttaaaacgctgacaaaaatctgataggaattaagaactttcgatttccaaaaatatcaataaaaagataggcattaatgactcgggcgaggtgatctttgtcacggaaaatttcgtcgtcttctgttacataatgccgattgtgatttcatagtgaacctatatactgatgaatgaatttacatatcagattccaagaaggagatgtagacaaacacagtgcaaaagagagtgccgccggcgctctcttttttgtgtgctgatcccggttataaaagacctgtgaaaagcgaccggtttgaaagggaaacacgacaattttcttaaccggtcagtgtataaagttttatagaaaatcaggaggatatatacatggttttggggttcatgtttattgtattcttttgaagggaataaaaactgacaaatttcgactgaagcaaaatttgaaaatgcatcaccttaccaattcgggatgggaaccgcacctcatgttcatgacctctttagaatatttcccttcatctttttaatctgcgcttaggtgaaaaagctgatcatgctgtgctgagcgtttcttctcgctatgacgctgctgtacatgcaaaaaaagtcctttaaatatcccagttgaatgacgatgaaagaggaaagaagaggaggaacagatcaattgataaaaaaagcggcaaacaaaaagttggttttgttttgtggaattgcggtgctttggatgtctttatttttaacgaatcataatgatgtacgcgccgatacgatcggcgagaaaatagcggaaactgccagacagcttgagggtgcgaaatacagctacggcggagagaagccgaaaacggggtttgactcgtcaggctttgtgcaatatgtgtttcaatcgctcgatattacgcttccgagaacggtaaaggaacaatcgactcttgggagcagt

SEQ ID NO: 17 - DNA, 651 bp, Bacillus licheniformis
atgaagaaatgggcatttgtatcagactttgatgggacgatttccaaacaggatttttactggatggtcattgataaatattttcccgaaggccgtgaattgttcaagaagtggaagtccggagaattaaaagatatcgaatttttgggaaccgtttttgcttcgattaatcaaagcgaacaaaaaatcattgatgacatccattccataccgattgatgaatatgtgcctgacttcattcagcatgtccagaaaagcggcggcgacttctacattttaagcgccggcacggattattacattcattatattttaaagaaatacgggattacagacgttgaggtctattcaaataaaggcttttttaaagaagacaatgttcatatggacattgatgagaatcattggcattactctgagcgctatgggattgataaatcaaaggtcattcaaaagctgaaagaagagtatgagacggtttattttgcaggcgacagtgaaccggattcgcacccggctaaatttgcggatgttacgtttgcaaaggatgcgctccaggatttgctgcgtcagcagggggtgccatttgtagccgttgaaacatttgaagacattgaacaatatcttaaagaaaaagggcggatcgtctaa

SEQ ID NO: 18 - DNA, 746 bp, Bacillus licheniformis
cctaagtgataatgattcgcattatcaatgtaaatatagcagatcaatccctctctcgtctatcactttttttgctaagtatgattagtgtggttttggttaatttgttactataaacagaaaaaggactgatgagagatggcagaaacgaacccggtgatcaaaaaattgcagttcaaggataatggacagcctgtactgattgtgaatccgcctgaggcatacagcggcgtcatcgctgaatttcaaggccctgttcatcatcacgccgaatcggaccaatatgattttgttcaggtattcgcagcgaccaacgcaaagctgcaggctttagccaaggaggctgaacgtcatttggcggaagacggtctgttttggctttgctacccgaaaaaatcatcgaaagtctacaaaggatcggactgcagccgcgatacagtagccggactgcttgcagaccagggctatgaaccggttcgccaaattgcaattgatgaagactggtctgcgctcagatttcgcaaggcggaaaacatcaaaacgatgaagcggaaatttgccgtaacagagaaaggtaagcagcgtacagatcaagaatgattatatacgcctcctttcagggggacgaatattcagcttgtgaacgaaagtacacaaaaaagaaataatattatgttcaatgattcacaaactttttgtataatgaatctaatcttttaaaataccatagaaaagaggtatgcagc

SEQ ID NO: 19 - DNA, 45 bp, Artificial Sequence
  nucleotide sequence of primer for amplifying homologous region 1 of dgp
agacagggccaacgaggcccctaagtgataagtattcgcattatc

SEQ ID NO: 20 - DNA, 37 bp, Artificial Sequence
  nucleotide sequence of primer for amplifying homologous region 1 of dgp
cggcattagacgatcgctgcatacctcttttctatgg

SEQ ID NO: 21 - DNA, 723 bp, Bacillus licheniformis
gatcgtctaatgccgcgccaggttaccagcatagccatccccgcggttttggacattagtgagggcgtgcttggccggttggatgagatattgagaaaacatcagtttgacaaggcgatcatgttttttgacgatttttcctatcagcagtatgagcattcactgaaaaccgcatttcaacatgttaaagttgaagccgttctgctgccgtccaatctggacatacaggagcttttgaagcgggcattttcgatcgggaattgcgatgtcattattgccatgggcggcgggtatgttgtggactgcggaaaatacatcgccttttccaagcggaccccgttcatcagcattccgacgtcggcatccaatgacgggtttgcgagcagcaattgctcgcttcaggtcgaaggaaaaaaaacaaccgttccggcaagggttccctacggaatcatagctgatttgagcattattcaaaaagcgccggattgctttattttggcggggatcggagatttgatgtccaatattacggccctttatgattgggagtttgaggagcggcacggggtcggcgatgtaaatgcgtttgcgtcgatgctcagcaagaaagcggtcaacagctttgtccgtacgccgatgcaggatattaaacagccgatcttcttaaaagagcttgtcagttctttgacaatgggcggcatcgctacggaaatcagcggaaac

SEQ ID NO: 22 - DNA, 33 bp, Artificial Sequence
  nucleotide sequence of primer for amplifying homologous region 2 of dgp
aaagaggtatgcagcgatcgtctaatgccgcgc

SEQ ID NO: 23 - DNA, 46 bp, Artificial Sequence
  nucleotide sequence of primer for amplifying homologous region 2 of dgp
agacagggccttattggccgtcaaagaactgacaagctcttttaag

SEQ ID NO: 24 - DNA, 1469 bp, Artificial Sequence
  nucleotide sequence comprising homologous region 1 and 2 of dgp
cctaagtgataatgattcgcattatcaatgtaaatatagcagatcaatccctctctcgtctatcactttttttgctaagtatgattagtgtggttttggttaatttgttactataaacagaaaaaggactgatgagagatggcagaaacgaacccggtgatcaaaaaattgcagttcaaggataatggacagcctgtactgattgtgaatccgcctgaggcatacagcggcgtcatcgctgaatttcaaggccctgttcatcatcacgccgaatcggaccaatatgattttgttcaggtattcgcagcgaccaacgcaaagctgcaggctttagccaaggaggctgaacgtcatttggcggaagacggtctgttttggctttgctacccgaaaaaatcatcgaaagtctacaaaggatcggactgcagccgcgatacagtagccggactgcttgcagaccagggctatgaaccggttcgccaaattgcaattgatgaagactggtctgcgctcagatttcgcaaggcggaaaacatcaaaacgatgaagcggaaatttgccgtaacagagaaaggtaagcagcgtacagatcaagaatgattatatacgcctcctttcagggggacgaatattcagcttgtgaacgaaagtacacaaaaaagaaataatattatgttcaatgattcacaaactttttgtataatgaatctaatcttttaaaataccatagaaaagaggtatgcagcgatcgtctaatgccgcgccaggttaccagcatagccatccccgcggttttggacattagtgagggcgtgcttggccggttggatgagatattgagaaaacatcagtttgacaaggcgatcatgttttttgacgatttttcctatcagcagtatgagcattcactgaaaaccgcatttcaacatgttaaagttgaagccgttctgctgccgtccaatctggacatacaggagcttttgaagcgggcattttcgatcgggaattgcgatgtcattattgccatgggcggcgggtatgttgtggactgcggaaaatacatcgccttttccaagcggaccccgttcatcagcattccgacgtcggcatccaatgacgggtttgcgagcagcaattgctcgcttcaggtcgaaggaaaaaaaacaaccgttccggcaagggttccctacggaatcatagctgatttgagcattattcaaaaagcgccggattgctttattttggcggggatcggagatttgatgtccaatattacggccctttatgattgggagtttgaggagcggcacggggtcggcgatgtaaatgcgtttgcgtcgatgctcagcaagaaagcggtcaacagctttgtccgtacgccgatgcaggatattaaacagccgatcttcttaaaagagcttgtcagttctttgacaatgggcggcatcgctacggaaatcagcggaaac

SEQ ID NO: 25 - DNA, 783 bp, Bacillus licheniformis
atgagtaaagtatctggaaaaattgcttttgttactggcggcggtcaaggaattggagaagcaatctgcaaacgattggcagaggacggattcgcagttgcagttgccgattataatgtagaaactgcaacacaagttgctgaggacatcaataagcttaacggcaaagcaattgcggttaaagtggatgttgctgatcgcgatgatgtttttaaagctgtcgatgaaacagtaaaacgtcttggcggtcttgatgtggtgattaataatgcgggtcttggaccaaccacccctattgaaagcattacatatgaagattatcggaaagtctatgatgttaacgttggcggtacttattggggaatacaagcagctgtaaaagcctttaaagaacttggacacggcgggaaaatcattaatgcatcttctcaagccggccaagtcggcaacccgggcttagcggtttacggaggaacaaagttcgctgttcgcgggattacccaaactgcggcaaaagatctagctgaattaggtattactgtaaacgccttttgtccgggtatcgttaaaactcctatgatgatggggattgcacagcaaaccgctgatgaagcaggcaagccgtttgaatggggcatggaacaattcgctaaaaatattgcattaaaacgcttatccgagccggaagatgtagcagcatgcgtttcttaccttgcagggccagattcagattatatgactggtcaagctcttatcattgatggcggaatggtatttaattaa

SEQ ID NO: 26 - DNA, 751 bp, Bacillus licheniformis
actccatgaactgacagtcggaaaatatggtgaagaaaaggcgaaatcattatggaattcactcggtttcggagctgaatccgtccttctcttaatcttagctgccgcttccggtcaagcgttcatgatgaacaggcggaaagagcatctgaaggcatttatgctcgcggtgttctatcactcttcttatttcgataaagcgcatgttttaaaaccataaccatacaaaaaaagcgggaggttttaacatgttatttatcataagaatggtgattattggcctattttcattgacagcaatcaatctgtttgtttttcaaggaattgaattcatgcacgcgattaccgatcttttcaatcgccaggacagctgaatttgaagcgatttgaaaaagctagacaataaaatttcatgaagcagtttgtttggcatgaatccggcattgtgcgggttcatgccttttcatttggtcttcatccgtttagcgatgactgaatcgctgttttatagcagaacatcccttttatagttttacatacagttcttcctccctctttcaaaaactattaaattttttcgaaaaattttaaacatattttcaacaaatgccgcggctttacttcaaatctacaaatataagatataatattcctgtaccaattaaataccaattacttatagaaagaagatgtttatatgagtaaagtatctggaaaaattgcttttgttactggcggcggtcaaggaatt

SEQ ID NO: 27 - DNA, 39 bp, Artificial Sequence
  nucleotide sequence of primer for amplifying homologous region 1 of budC
agacagggccaacgaggccactccatgaactgacagtcg

SEQ ID NO: 28 - DNA, 39 bp, Artificial Sequence
  nucleotide sequence of primer for amplifying homologous region 1 of budC
catcaatgataagagaattccttgaccgccgccagtaac

SEQ ID NO: 29 - DNA, 776 bp, Bacillus licheniformis
ctcttatcattgatggcggaatggtatttaattaattttaaaattatattctatatggagggaggagttttcccctccatatttagtattgaataatcagctatatagcatggcttaaaaccgtgtaatacgaaacggccacggcgtccaaccacgccttgatttatggttcacgtttaaaaaacaaagaacgcaggccgttggttcctcccccatcggcaaatcgtggcgtccatgaatttcgaatcgcatcaatacttagcgtttactgccaaattgtcattctaaacgcccttcttcttgaagttttcccaattttttatgattgcccaggtccctttatctgttgaaggacggctccatcatttaggatataacgaagcgggacaattgagcggaaatgatacaaacaagaggctaattttaattaaaaaaaggccgaagtgagcaacttcgccctcaagcaaggcgccgtgaggaaatccatatgtttacgatcttttgaacccctgtttcaaaatgcactagtgcgaggatttcccctgcgataagcggcacccaagatatcttctttgaattctactccaagcctccataggttttatttacgcgctttttccgtcaactcgtttattttctccatttttttcgatttcctctaaactgcgacctcgagtttcagggacgcgtgtccggataaatacaactccaagcaaacaaatcacaccgaagattgcaaacacagcttcttgagacatcgaagcggtcataacagg

SEQ ID NO: 30 - DNA, 38 bp, Artificial Sequence
  nucleotide sequence of primer for amplifying homologous region 2 of budC
ggcggtcaaggaattctcttatcattgatggcggaatg

SEQ ID NO: 31 - DNA, 40 bp, Artificial Sequence
  nucleotide sequence of primer for amplifying homologous region 2 of budC
agacagggccttattggcccctgttatgaccgcttcgatg

SEQ ID NO: 32 - DNA, 1527 bp, Artificial Sequence
  nucleotide sequence comprising homologous region 1 and 2 of budC
actccatgaactgacagtcggaaaatatggtgaagaaaaggcgaaatcattatggaattcactcggtttcggagctgaatccgtccttctcttaatcttagctgccgcttccggtcaagcgttcatgatgaacaggcggaaagagcatctgaaggcatttatgctcgcggtgttctatcactcttcttatttcgataaagcgcatgttttaaaaccataaccatacaaaaaaagcgggaggttttaacatgttatttatcataagaatggtgattattggcctattttcattgacagcaatcaatctgtttgtttttcaaggaattgaattcatgcacgcgattaccgatcttttcaatcgccaggacagctgaatttgaagcgatttgaaaaagctagacaataaaatttcatgaagcagtttgtttggcatgaatccggcattgtgcgggttcatgccttttcatttggtcttcatccgtttagcgatgactgaatcgctgttttatagcagaacatcccttttatagttttacatacagttcttcctccctctttcaaaaactattaaattttttcgaaaaattttaaacatattttcaacaaatgccgcggctttacttcaaatctacaaatataagatataatattcctgtaccaattaaataccaattacttatagaaagaagatgtttatatgagtaaagtatctggaaaaattgcttttgttactggcggcggtcaaggaattctcttatcattgatggcggaatggtatttaattaattttaaaattatattctatatggagggaggagttttcccctccatatttagtattgaataatcagctatatagcatggcttaaaaccgtgtaatacgaaacggccacggcgtccaaccacgccttgatttatggttcacgtttaaaaaacaaagaacgcaggccgttggttcctcccccatcggcaaatcgtggcgtccatgaatttcgaatcgcatcaatacttagcgtttactgccaaattgtcattctaaacgcccttcttcttgaagttttcccaattttttatgattgcccaggtccctttatctgttgaaggacggctccatcatttaggatataacgaagcgggacaattgagcggaaatgatacaaacaagaggctaattttaattaaaaaaaggccgaagtgagcaacttcgccctcaagcaaggcgccgtgaggaaatccatatgtttacgatcttttgaacccctgtttcaaaatgcactagtgcgaggatttcccctgcgataagcggcacccaagatatcttctttgaattctactccaagcctccataggttttatttacgcgctttttccgtcaactcgtttattttctccatttttttcgatttcctctaaactgcgacctcgagtttcagggacgcgtgtccggataaatacaactccaagcaaacaaatcacaccgaagattgcaaacacagcttcttgagacatcgaagcggtcataacagg

SEQ ID NO: 33 - DNA, 1104 bp, Bacillus licheniformis
atgtcaaaatcagtaaaatcagtcacatcacctaaaaaatttattacaggaaaacgactgctggagaacttgaacgactacattgaagattttggcgacaacgcatatatcatttgcgatgaattcattttggaacgcgctcaaaaagaagcggggaattcgattcagaaagccggcaatcaagccgtttttgaaaaattcaattacgaatgcacacaggaagaaatcgatcgcaaccgggagcttgcacgcaatgcaggcgctaatatcatcgttgggatcggaggcggtaaaacgcttgataccgcaaaagccaccgcttattacgagaagctgccggttgtgattttcccgacaattgcttctacggatgctccatgtacggcccttgccgtcatttataaacacgacggatcgtttgaccgctatctgtttttgccgacgaacccagatgtcgttcttgcggactctgagattttggcatccgcgccgccgcgctttttcgcagccggtatcggtgacgccttggcgacgtattttgaagcgcgcgcctgctttaaagcaaacggcgataacctcgtgctgatgaagccttcaacaactggattgggacttgcccgtctttgctatgatacgctgttggaaaacggtgtgaaagcgatgcaggcggttaagcacggcgtttccacacgagcggtcgaagatacaatcgaggcgaccatctatttaagcggcgtcggtgccgaatcaggcggtcttgccgccgcacacgcgatccacaacggaatgacagccgttccttctctgcacagggctcagcacggcgaaaaagtcacgttcggccttttggcgcagcttgttcttgaaaacgcgccggccgaagaattggagaccgttattgactttatcaaaggcgtcggtcttccgttgacattaaaagacctcggagtcgacgaatttgtcgaagaagaatggcgccaagtcgctcaaagcgcttgcgcggaaggcgacacaatgggcaacatgccgttcccagtcacccctgacgacgtctacaatgcgatcgtcgccgccaacgcgattgcagaatcttatcacgattaa

SEQ ID NO: 34 - DNA, 910 bp, Bacillus licheniformis
aatgctgaagcgatttccaacaaggcgatccattggggtttttcaaaaagcaaaaaccatcagccggcagatgcgggtcaagagctgaacaaccttttacagcagtacgacgccttttatttgggcaacacaaaggaaaaaacgatctatctgacctttgataacggctatgaaaacggctacacccctcaggtgctcgatgttctgaaaaaacaaaacgtcaaagcggccttttttgtgacgggccattttgtcaaagatcagccggagctgatcaagcgaatggccgaggaggggcatatcatcgggaatcattcatatcaccatccggatctgacgacgaaaacaagccgcgtcattcaagaggaattggaatcggtcgatgaggaggtttacaaaatcacaggcgaaaaaaacaacctctacctgagaccgcctcggggcattttcagcgagcgggtgctcgaagaaacgaaaaagctcggctatcaaacggtattctggtctgttgcttttgtcgattggaaaatcaatgcccaaaaagggtggcgctatgcgtacgacaatatgatgaaacaggctcaccccggcgccatctatctgcttcacaccgtctcgagagacaatgccgaagcgcttgatcaggcgatcaccgacttgaaaaaagaaggttatacatttaaaagcctcgatgacctgatgtttgaaaaatctatgatgcttgagaccctttgaaagaacaatgccccggccgctttgccggggttttgctttggctgaaaaaattgatgcttcaggctctttttatttcccctagtcaattctatagaataaaaatccattttatatacatatattactagatttaaaaagaaaataggtatatcattgatagtgaaggggaattacc

SEQ ID NO: 35 - DNA, 49 bp, Artificial Sequence
  nucleotide sequence of primer for amplifying homologous region 1 of gdh
agacagggccaacgaggccaatgctgaagcgatttccaacaaggcgatc

SEQ ID NO: 36 - DNA, 35 bp, Artificial Sequence
  nucleotide sequence of primer for amplifying homologous region 1 of gdh
acggcttttcgtctaggtaattccccttcactatc

SEQ ID NO: 37 - DNA, 886 bp, Bacillus licheniformis
tagacgaaaagccgtttccgtgaaggagcggctttctgctttgggttagtatattagtttgtgaatcggcggtctgtccgtgcttttgaatatgaattgtgtggtacgtttcccagagtaaaattatgaatttcttttatagcagtttcccaaaaacgagctgtttgactcgtgtgacagccgttcatttcaccactttaatcttcaacctcggctcttcttcaattccggatgcaaatgcatcctcatttcccggagccgtaaaggtgacgctgtacgtttcctgtgaatgcggcgacagttccagctcttccggctgaaagtcaaattcatttattatatcaggggtgagctggacgcgttcggtctttttcccgtagttgttgactttcacctcacagtccatgcttcctgcttccatatcgccctgatagctgcaagcgcttccccttttcatatattccacggcgctatcgccttgtgcattccatttttgaaagaacatcagctgttctgtgaccagcgggtaaaatactgaaataccgatgataaacaaaaacagcttaaagcggatccacggtactccataataatggcgccacgccataatgaagccggcgatgatcataaacatgcagatcagaaccactaaattccggatgggcagttttaaaaagcccgaaagcgcgtctgctacagacgcgccttgatgattctcggcgctgatcaacaggccgataacaatcatgatgatgccggcaagccctgtatgtaccttcatttctttccctcctcagttgtagaaatagtcgaacagagaggaaaaaggtttccggttttacttgaaaatgtcaaaccatcctttatgccggaaccagaagatcat

SEQ ID NO: 38 - DNA, 40 bp, Artificial Sequence
  nucleotide sequence of primer for amplifying homologous region 2 of gdh
tgaaggggaattacctagacgaaaagccgtttccgtgaag

SEQ ID NO: 39 - DNA, 38 bp, Artificial Sequence
  nucleotide sequence of primer for amplifying homologous region 2 of gdh
agacagggccttattggccatgatcttctggttccggc

SEQ ID NO: 40 - DNA, 1796 bp, Artificial Sequence
  nucleotide sequence comprising homologous region 1 and 2 of gdh
aatgctgaagcgatttccaacaaggcgatccattggggtttttcaaaaagcaaaaaccatcagccggcagatgcgggtcaagagctgaacaaccttttacagcagtacgacgccttttatttgggcaacacaaaggaaaaaacgatctatctgacctttgataacggctatgaaaacggctacacccctcaggtgctcgatgttctgaaaaaacaaaacgtcaaagcggccttttttgtgacgggccattttgtcaaagatcagccggagctgatcaagcgaatggccgaggaggggcatatcatcgggaatcattcatatcaccatccggatctgacgacgaaaacaagccgcgtcattcaagaggaattggaatcggtcgatgaggaggtttacaaaatcacaggcgaaaaaaacaacctctacctgagaccgcctcggggcattttcagcgagcgggtgctcgaagaaacgaaaaagctcggctatcaaacggtattctggtctgttgcttttgtcgattggaaaatcaatgcccaaaaagggtggcgctatgcgtacgacaatatgatgaaacaggctcaccccggcgccatctatctgcttcacaccgtctcgagagacaatgccgaagcgcttgatcaggcgatcaccgacttgaaaaaagaaggttatacatttaaaagcctcgatgacctgatgtttgaaaaatctatgatgcttgagaccctttgaaagaacaatgccccggccgctttgccggggttttgctttggctgaaaaaattgatgcttcaggctctttttatttcccctagtcaattctatagaataaaaatccattttatatacatatattactagatttaaaaagaaaataggtatatcattgatagtgaaggggaattacctagacgaaaagccgtttccgtgaaggagcggctttctgctttgggttagtatattagtttgtgaatcggcggtctgtccgtgcttttgaatatgaattgtgtggtacgtttcccagagtaaaattatgaatttcttttatagcagtttcccaaaaacgagctgtttgactcgtgtgacagccgttcatttcaccactttaatcttcaacctcggctcttcttcaattccggatgcaaatgcatcctcatttcccggagccgtaaaggtgacgctgtacgtttcctgtgaatgcggcgacagttccagctcttccggctgaaagtcaaattcatttattatatcaggggtgagctggacgcgttcggtctttttcccgtagttgttgactttcacctcacagtccatgcttcctgcttccatatcgccctgatagctgcaagcgcttccccttttcatatattccacggcgctatcgccttgtgcattccatttttgaaagaacatcagctgttctgtgaccagcgggtaaaatactgaaataccgatgataaacaaaaacagcttaaagcggatccacggtactccataataatggcgccacgccataatgaagccggcgatgatcataaacatgcagatcagaaccactaaattccggatgggcagttttaaaaagcccgaaagcgcgtctgctacagacgcgccttgatgattctcggcgctgatcaacaggccgataacaatcatgatgatgccggcaagccctgtatgtaccttcatttctttccctcctcagttgtagaaatagtcgaacagagaggaaaaaggtttccggttttacttgaaaatgtcaaaccatcctttatgccggaaccagaagatcat